European Patent Application EP 4 130 029 A1, published February 8, 2023. Title: Pharmaceutical Compositions Comprising HLA Fusion Proteins. Applicant: ImmunOs Therapeutics AG. The sequence listing filed with the application follows.

SEQUENCE LISTING (6 sequences)

SEQ ID NO: 1 - protein, 280 aa, Artificial Sequence
  HLA-B57:01 extracellular domain A46E V97R
GSHSMRYFYTAMSRPGRGEPRFIAVGYVDDTQFVRFDSDAASPRMEPRAPWIEQEGPEYWDGETRNMKASAQTYRENLRIALRYYNQSEAGSHIIQRMYGCDVGPDGRLLRGHDQSAYDGKDYIALNEDLSSWTAADTAAQITQRKWEAARVAEQLRAYLEGLCVEWLRRYLENGKETLQRADPPKTHVTHHPISDHEATLRCWALGFYPAEITLTWQRDGEDQTQDTELVETRPAGDRTFQKWAAVVVPSGEEQRYTCHVQHEGLPKPLTLRWEPSSQS

SEQ ID NO: 2 - protein, 228 aa, Artificial Sequence
  Optimized IgG4 Fc
ESKYGPPCPPCPAPEFLGGPSVFLFPPKPKDTLMISRTPEVTCVVVDVSQEDPEVQFNWYVDGVEVHNAKTKPREEQFNSTYRVVSVLTVLHQDWLNGKEYKCKVSNKGLPSSIEKTISKAKGQPREPQVYTLPPSQEEMTKNQVSLTCLVKGFYPSDIAVEWESNGQPENNYKTTPPVLDSDGSFFLYSRLTVDKSRWQEGNVFSCSVMHEALHNHYTQKSLSLSLG

SEQ ID NO: 3 - protein, 10 aa, Artificial Sequence
  peptide linker
GGGGSGGGGS

SEQ ID NO: 4 - protein, 21 aa, Artificial sequence
  HLA fusion protein secretory signal
AAAMNFGLRLIFLVLTLKGVQ

SEQ ID NO: 5 - protein, 518 aa, Artificial sequence
  variant HLA-B57 extracellular domain IgG4 Fc fusion protein, lacking secretory signal
GSHSMRYFYTAMSRPGRGEPRFIAVGYVDDTQFVRFDSDAASPRMEPRAPWIEQEGPEYWDGETRNMKASAQTYRENLRIALRYYNQSEAGSHIIQRMYGCDVGPDGRLLRGHDQSAYDGKDYIALNEDLSSWTAADTAAQITQRKWEAARVAEQLRAYLEGLCVEWLRRYLENGKETLQRADPPKTHVTHHPISDHEATLRCWALGFYPAEITLTWQRDGEDQTQDTELVETRPAGDRTFQKWAAVVVPSGEEQRYTCHVQHEGLPKPLTLRWEPSSQSGGGGSGGGGSESKYGPPCPPCPAPEFLGGPSVFLFPPKPKDTLMISRTPEVTCVVVDVSQEDPEVQFNWYVDGVEVHNAKTKPREEQFNSTYRVVSVLTVLHQDWLNGKEYKCKVSNKGLPSSIEKTISKAKGQPREPQVYTLPPSQEEMTKNQVSLTCLVKGFYPSDIAVEWESNGQPENNYKTTPPVLDSDGSFFLYSRLTVDKSRWQEGNVFSCSVMHEALHNHYTQKSLSLSLG

SEQ ID NO: 6 - protein, 99 aa, Homo sapiens [sequence omitted]